European Patent Application EP 4 748 851 A1, published May 27, 2026. Title: 一种角蛋白CF5、制法和其药物组合物与用途. Applicant: 中国医学科学院药物研究所. The sequence listing filed with the application follows.

SEQUENCE LISTING (2 sequences)

SEQ ID NO: 1 - protein, 461 aa, unidentified
MASQICSPIFSSGSVRGLCGTAGGITRVSSVRSVGSCRVPSLAGAARSGSSVRLGLSGFGSCLPASCLSTGYYPSSFVGSGGWFYEGSFNGNEKETMQFLNDRLANYLEKVRQLEQENAELESRIREWYESQIPYICPDYQSYFRTIEELQQKILLTKAENARLVLQIDNAKLAADDFRTKYETELGLRQLVEADTNGLRRILDELTLCKADLEMQVESLKEELLCLKKNHEEEVNVLRGQLGDRLNVEVDAAPSVDLNKILDDMRCQYETLVENNRRDVEAWFNTQTEELNQQVVSSSEQLQSCQVEIIELRRTVNALEIELQAQQSTRNSLESTLAETEARYSSQLAQMQGLITNVEAQLAEIRCDLERQNHEYQVLLDVKARLESEIATYRRLLESEDCKLPAHPCATECKPAIRVPYVSTVPCAQASQVSAQIRTITEEIRDGKIISSREHLQPCPL

SEQ ID NO: 2 - DNA, 1383 bp, unidentified
  source 1..1383: mol_type = other DNA
atggcgagccagatttgcagcccgatttttagcagcggcagcgtgcgcggtttatgcggcaccgcgggtggtattactcgtgtgagcagcgttcgtagcgtgggcagctgtcgtgttcctagcttggcgggtgcggcgcgttcaggcagcagcgttcgtttaggactgagcggttttggcagctgcttacctgcgagctgtctgagcactggttattatccgagcagctttgtgggcagcggcggctggttttatgaaggcagctttaacggcaacgaaaaagaaaccatgcagtttctgaacgaccgcctggcgaactatctggaaaaagtgcgccagctggaacaggaaaacgcggaactggaaagccgcattcgcgaatggtatgaaagccagattccgtatatttgcccggattatcagagctattttcgcaccattgaagagctgcagcagaaaattctgctgaccaaagcggaaaacgcgcgcctggtgttacagattgataacgcgaaactggcggcggatgattttcgcaccaaatatgaaaccgaactgggcctgcgccagctggtggaagcggatactaatggcttacgtcgcattctggatgaactgaccttatgcaaagcggatctggaaatgcaggtggaaagcctgaaagaagaactgctgtgcctgaaaaaaaaccacgaagaagaagtgaacgtgctgcgcggccagctgggtgatcgtttaaatgttgaagtggatgcggcgcctagcgtggatttaaacaaaattctggatgacatgcgctgccagtatgaaaccctggtggaaaacaaccgccgcgatgtggaagcgtggtttaacacccagaccgaagaactgaaccagcaggtggtgagcagcagcgaacagctgcaaagctgtcaagtggaaattattgaactgcgccgcaccgtgaacgcgctggaaattgaactgcaggcgcagcagagcacccgcaatagcttagaaagcaccctggcggaaaccgaagcgcgctatagcagccaattagcgcagatgcaaggcctgattaccaacgtggaagcgcagctggcggaaattcgctgcgatctggaacgccagaaccatgaatatcaggtgctgctggatgtgaaagcgcgcctggaaagcgaaattgcgacctatcgccgcctgctggaaagcgaagattgcaaactgccggcgcatccgtgcgcgactgaatgtaaacctgcgattcgcgtgccgtatgtgagcaccgttccgtgcgcgcaagcgtcacaggttagcgcgcaaattcgtaccattaccgaagaaattcgcgatggcaaaattatcagcagccgcgaacatctgcagccgtgcccttta